European Patent Specification EP 4 274 838 B1, published September 25, 2024. Title: BICYCLIC PEPTIDE LIGANDS SPECIFIC FOR NK CELLS. Applicant: BicycleTx Limited. The sequence listing filed with the application follows.

SEQUENCE LISTING (268 sequences)

SEQ ID NO: 1 - protein, 12 aa, Artificial
  Synthetic Peptide
CNLQKPCMKYPC

SEQ ID NO: 2 - protein, 12 aa, Artificial
  Synthetic Peptide
CNLQNPCMKFPC

SEQ ID NO: 3 - protein, 14 aa, Artificial
  Synthetic Peptide
CNLQAPCMQTGKVC

SEQ ID NO: 4 - protein, 14 aa, Artificial
  Synthetic Peptide
CNLQAPCMLTGKVC

SEQ ID NO: 5 - protein, 15 aa, Artificial
  Synthetic Peptide
CLLHDHCPNTHPKLC

SEQ ID NO: 6 - protein, 15 aa, Artificial
  Synthetic Peptide
CLLHEHCPNTHPKMC

SEQ ID NO: 7 - protein, 15 aa, Artificial
  Synthetic Peptide
CLLHDHCPNSHPEIC

SEQ ID NO: 8 - protein, 15 aa, Artificial
  Synthetic Peptide
CLLHDHCPNTHPIIC

SEQ ID NO: 9 - protein, 13 aa, Artificial
  Synthetic Peptide
CYLPDWLCGDEYC

SEQ ID NO: 10 - protein, 13 aa, Artificial
  Synthetic Peptide
CYLPDYLCGDEYC

SEQ ID NO: 11 - protein, 13 aa, Artificial
  Synthetic Peptide
CDLTTHNCQWGIC

SEQ ID NO: 12 - protein, 13 aa, Artificial
  Synthetic Peptide
CYLPDYLCGDEYC

SEQ ID NO: 13 - protein, 13 aa, Artificial
  Synthetic Peptide
CYLPDWLCGDEYC

SEQ ID NO: 14 - protein, 13 aa, Artificial
  Synthetic Peptide
  Xaa (2)..(2): Xaa is 2,6DiMeTyr
CXLPDYLCGDEYC

SEQ ID NO: 15 - protein, 13 aa, Artificial
  Synthetic Peptide
  Xaa (3)..(3): Xaa is tBuAla
CYXPDYLCGDEYC

SEQ ID NO: 16 - protein, 13 aa, Artificial
  Synthetic Peptide
  Xaa (3)..(3): Xaa is Cba
CYXPDYLCGDEYC

SEQ ID NO: 17 - protein, 13 aa, Artificial
  Synthetic Peptide
  Xaa (4)..(4): Xaa is HyP
CYLXDYLCGDEYC

SEQ ID NO: 18 - protein, 13 aa, Artificial
  Synthetic Peptide
  Xaa (4)..(4): Xaa is Aze
CYLXDYLCGDEYC

SEQ ID NO: 19 - protein, 13 aa, Artificial
  Synthetic Peptide
  Xaa (4)..(4): Xaa is Aib
CYLXDYLCGDEYC

SEQ ID NO: 20 - protein, 13 aa, Artificial
  Synthetic Peptide
  Xaa (6)..(6): Xaa is 1Nal
CYLPDXLCGDEYC

SEQ ID NO: 21 - protein, 13 aa, Artificial
  Synthetic Peptide
  Xaa (6)..(6): Xaa is 2Nal
CYLPDXLCGDEYC

SEQ ID NO: 22 - protein, 13 aa, Artificial
  Synthetic Peptide
  Xaa (6)..(6): Xaa is 3Pal
CYLPDXLCGDEYC

SEQ ID NO: 23 - protein, 13 aa, Artificial
  Synthetic Peptide
  Xaa (6)..(6): Xaa is 2,6DiMeTyr
CYLPDXLCGDEYC

SEQ ID NO: 24 - protein, 13 aa, Artificial
  Synthetic Peptide
  Xaa (6)..(6): Xaa is tBuAla
  misc_feature (7)..(7): Xaa can be any naturally occurring amino acid
CYLPDWXCGDEYC

SEQ ID NO: 25 - protein, 13 aa, Artificial
  Synthetic Peptide
  Xaa (7)..(7): Xaa is Cba
CYLPDWXCGDEYC

SEQ ID NO: 26 - protein, 13 aa, Artificial
  Synthetic Peptide
CYLPDYLCADEYC

SEQ ID NO: 27 - protein, 13 aa, Artificial
  Synthetic Peptide
  Xaa (12)..(12): Xaa is 2,6DiMeTyr
CYLPDYLCGDEXC

SEQ ID NO: 28 - protein, 13 aa, Artificial
  Synthetic Peptide
CALPDYLCGDEYC

SEQ ID NO: 29 - protein, 13 aa, Artificial
  Synthetic Peptide
CYAPDYLCGDEYC

SEQ ID NO: 30 - protein, 13 aa, Artificial
  Synthetic Peptide
CYLADYLCGDEYC

SEQ ID NO: 31 - protein, 13 aa, Artificial
  Synthetic Peptide
CYLPAYLCGDEYC

SEQ ID NO: 32 - protein, 13 aa, Artificial
  Synthetic Peptide
CYLPDALCGDEYC

SEQ ID NO: 33 - protein, 13 aa, Artificial
  Synthetic Peptide
CYLPDYACGDEYC

SEQ ID NO: 34 - protein, 13 aa, Artificial
  Synthetic Peptide
CYLPDYLCADEYC

SEQ ID NO: 35 - protein, 13 aa, Artificial
  Synthetic Peptide
CYLPDYLCGAEYC

SEQ ID NO: 36 - protein, 13 aa, Artificial
  Synthetic Peptide
CYLPDYLCGDAYC

SEQ ID NO: 37 - protein, 13 aa, Artificial
  Synthetic Peptide
CYLPDYLCGDEAC

SEQ ID NO: 38 - protein, 13 aa, Artificial
  Synthetic Peptide
  Xaa (3)..(3): Xaa is C5A
CYXPDYLCGDEYC

SEQ ID NO: 39 - protein, 13 aa, Artificial
  Synthetic Peptide
  Xaa (3)..(3): Xaa is Cha
CYXPDYLCGDEYC

SEQ ID NO: 40 - protein, 13 aa, Artificial
  Synthetic Peptide
  Xaa (3)..(3): Xaa is Cba
CYXPDYLCADEYC

SEQ ID NO: 41 - protein, 13 aa, Artificial
  Synthetic Peptide
  Xaa (6)..(6): Xaa is 4FPhe
CYLPDXLCGDEYC

SEQ ID NO: 42 - protein, 13 aa, Artificial
  Synthetic Peptide
  Xaa (6)..(6): Xaa is 4MeOPhe
CYLPDXLCGDEYC

SEQ ID NO: 43 - protein, 13 aa, Artificial
  Synthetic Peptide
  Xaa (6)..(6): Xaa is NO2Phe
CYLPDXLCGDEYC

SEQ ID NO: 44 - protein, 13 aa, Artificial
  Synthetic Peptide
  Xaa (6)..(6): Xaa is 4MePhe
CYLPDXLCGDEYC

SEQ ID NO: 45 - protein, 13 aa, Artificial
  Synthetic Peptide
  Xaa (6)..(6): Xaa is pCoPhe
CYLPDXLCGDEYC

SEQ ID NO: 46 - protein, 13 aa, Artificial
  Synthetic Peptide
  misc_feature (6)..(6): Xaa can be any naturally occurring amino acid
CYLPDXLCGDEYC

SEQ ID NO: 47 - protein, 13 aa, Artificial
  Synthetic Peptide
  Xaa (6)..(6): Xaa is 4tBuPhe
CYLPDXLCGDEYC

SEQ ID NO: 48 - protein, 13 aa, Artificial
  Synthetic Peptide
  Xaa (6)..(6): Xaa is CF3Phe
CYLPDXLCGDEYC

SEQ ID NO: 49 - protein, 13 aa, Artificial
  Synthetic Peptide
  Xaa (6)..(6): Xaa is 4CNPhe
CYLPDXLCGDEYC

SEQ ID NO: 50 - protein, 13 aa, Artificial
  Synthetic Peptide
  Xaa (6)..(6): Xaa is 4ClPhe
CYLPDXLCGDEYC

SEQ ID NO: 51 - protein, 13 aa, Artificial
  Synthetic Peptide
  Xaa (6)..(6): Xaa is HPhe
CYLPDXLCGDEYC

SEQ ID NO: 52 - protein, 13 aa, Artificial
  Synthetic Peptide
  Xaa (2)..(2): Xaa is 2,6DiMeTyr
CXLPDWLCGDEYC

SEQ ID NO: 53 - protein, 13 aa, Artificial
  Synthetic Peptide
  Xaa (3)..(3): Xaa is Cba
CYXPDWLCGDEYC

SEQ ID NO: 54 - protein, 13 aa, Artificial
  Synthetic Peptide
  Xaa (4)..(4): Xaa is Aze
CYLXDWLCGDEYC

SEQ ID NO: 55 - protein, 13 aa, Artificial
  Synthetic Peptide
CYLPDWLCADEYC

SEQ ID NO: 56 - protein, 13 aa, Artificial
  Synthetic Peptide
CSLPDYLCGDEYC

SEQ ID NO: 57 - protein, 13 aa, Artificial
  Synthetic Peptide
CDLTTHNCQWGIC

SEQ ID NO: 58 - protein, 13 aa, Artificial
  Synthetic Peptide
CDLTTHNCLWGVC

SEQ ID NO: 59 - protein, 13 aa, Artificial
  Synthetic Peptide
CNLQLHNCIWGVC

SEQ ID NO: 60 - protein, 12 aa, Artificial
  Synthetic Peptide
CPPTVYCHPLDC

SEQ ID NO: 61 - protein, 13 aa, Artificial
  Synthetic Peptide
CRWSVEDPCGAWC

SEQ ID NO: 62 - protein, 14 aa, Artificial
  Synthetic Peptide
CVGLEELGPCSDLC

SEQ ID NO: 63 - protein, 14 aa, Artificial
  Synthetic Peptide
CNLQQACLHTGKVC

SEQ ID NO: 64 - protein, 14 aa, Artificial
  Synthetic Peptide
CNLQAACMLTGKVC

SEQ ID NO: 65 - protein, 14 aa, Artificial
  Synthetic Peptide
CNLQAPCMATGKVC

SEQ ID NO: 66 - protein, 14 aa, Artificial
  Synthetic Peptide
CNLQAPCMLAGKVC

SEQ ID NO: 67 - protein, 14 aa, Artificial
  Synthetic Peptide
CNLQAPCMLTAKVC

SEQ ID NO: 68 - protein, 14 aa, Artificial
  Synthetic Peptide
CNLQAPCMLTGAVC

SEQ ID NO: 69 - protein, 14 aa, Artificial
  Synthetic Peptide
CNLQAPCMLTGKAC

SEQ ID NO: 70 - protein, 14 aa, Artificial
  Synthetic Peptide
  Xaa (3)..(3): Xaa is tBuAla
CNXQAPCMLTGKVC

SEQ ID NO: 71 - protein, 14 aa, Artificial
  Synthetic Peptide
  Xaa (6)..(6): Xaa is Sar
CNLQAXCMLTGKVC

SEQ ID NO: 72 - protein, 14 aa, Artificial
  Synthetic Peptide
  Xaa (6)..(6): Xaa is Cis-HyP
CNLQAXCMLTGKVC

SEQ ID NO: 73 - protein, 14 aa, Artificial
  Synthetic Peptide
  Xaa (6)..(6): Xaa is HyP
CNLQAXCMLTGKVC

SEQ ID NO: 74 - protein, 14 aa, Artificial
  Synthetic Peptide
  Xaa (6)..(6): Xaa is NMeAla
CNLQAXCMLTGKVC

SEQ ID NO: 75 - protein, 14 aa, Artificial
  Synthetic Peptide
CNLQAPCLLTGKVC

SEQ ID NO: 76 - protein, 14 aa, Artificial
  Synthetic Peptide
  Xaa (8)..(8): Xaa is Nle
CNLQAPCXLTGKVC

SEQ ID NO: 77 - protein, 14 aa, Artificial
  Synthetic Peptide
  Xaa (8)..(8): Xaa is Cba
CNLQAPCXLTGKVC

SEQ ID NO: 78 - protein, 14 aa, Artificial
  Synthetic Peptide
CNLQAPCMETGKVC

SEQ ID NO: 79 - protein, 14 aa, Artificial
  Synthetic Peptide
CNLQAPCMFTGKVC

SEQ ID NO: 80 - protein, 14 aa, Artificial
  Synthetic Peptide
CNLQAPCMYTGKVC

SEQ ID NO: 81 - protein, 14 aa, Artificial
  Synthetic Peptide
  Xaa (9)..(9): Xaa is Cba
CNLQAPCMXTGKVC

SEQ ID NO: 82 - protein, 14 aa, Artificial
  Synthetic Peptide
  Xaa (9)..(9): Xaa is tBuAla
CNLQAPCMXTGKVC

SEQ ID NO: 83 - protein, 14 aa, Artificial
  Synthetic Peptide
  Xaa (9)..(9): Xaa is Cha
CNLQAPCMXTGKVC

SEQ ID NO: 84 - protein, 14 aa, Artificial
  Synthetic Peptide
CNLQAPCMLTAKVC

SEQ ID NO: 85 - protein, 14 aa, Artificial
  Synthetic Peptide
CNLQAPCMLTGRVC

SEQ ID NO: 86 - protein, 14 aa, Artificial
  Synthetic Peptide
  Xaa (12)..(12): Xaa is Agb
CNLQAPCMLTGXVC

SEQ ID NO: 87 - protein, 14 aa, Artificial
  Synthetic Peptide
  Xaa (13)..(13): Xaa is tBuGly
CNLQAPCMLTGKXC

SEQ ID NO: 88 - protein, 14 aa, Artificial
  Synthetic Peptide
  Xaa (13)..(13): Xaa is Chg
CNLQAPCMLTGKXC

SEQ ID NO: 89 - protein, 14 aa, Artificial
  Synthetic Peptide
  Xaa (13)..(13): Xaa is Cbg
CNLQAPCMLTGKXC

SEQ ID NO: 90 - protein, 14 aa, Artificial
  Synthetic Peptide
  Xaa (12)..(12): Xaa is HArg
CNLQAPCMLTGXVC

SEQ ID NO: 91 - protein, 14 aa, Artificial
  Synthetic Peptide
  Xaa (6)..(6): Xaa is Aze
CNLQAXCMLTGKVC

SEQ ID NO: 92 - protein, 14 aa, Artificial
  Synthetic Peptide
  Xaa (6)..(6): Xaa is Pip
CNLQAXCMLTGKVC

SEQ ID NO: 93 - protein, 14 aa, Artificial
  Synthetic Peptide
CNLQAPCMVTGKVC

SEQ ID NO: 94 - protein, 14 aa, Artificial
  Synthetic Peptide
  Xaa (9)..(9): Xaa is Nle
CNLQAPCMXTGKVC

SEQ ID NO: 95 - protein, 14 aa, Artificial
  Synthetic Peptide
  Xaa (9)..(9): Xaa is Nva
CNLQAPCMXTGKVC

SEQ ID NO: 96 - protein, 14 aa, Artificial
  Synthetic Peptide
  Xaa (13)..(13): Xaa is AlloIle
CNLQAPCMLTGKXC

SEQ ID NO: 97 - protein, 14 aa, Artificial
  Synthetic Peptide
  Xaa (13)..(13): Xaa is EPA
CNLQAPCMLTGKXC

SEQ ID NO: 98 - protein, 14 aa, Artificial
  Synthetic Peptide
CNLQQPCMLTGKVC

SEQ ID NO: 99 - protein, 14 aa, Artificial
  Synthetic Peptide
  misc_feature (6)..(6): Xaa can be any naturally occurring amino acid
CNLQAXCMLTGKVC

SEQ ID NO: 100 - protein, 14 aa, Artificial
  Synthetic Peptide
CNLQAPCMHTGKVC

SEQ ID NO: 101 - protein, 14 aa, Artificial
  Synthetic Peptide
CNLQAPCLHTGKVC

SEQ ID NO: 102 - protein, 14 aa, Artificial
  Synthetic Peptide
CNLQQACMQTGKVC

SEQ ID NO: 103 - protein, 15 aa, Artificial
  Synthetic Peptide
CLLHDHCPNTHPKMC

SEQ ID NO: 104 - protein, 13 aa, Artificial
  Synthetic Peptide
CDLTTHNCIWGVC

SEQ ID NO: 105 - protein, 13 aa, Artificial
  Synthetic Peptide
CNLQLHNCIWGVC

SEQ ID NO: 106 - protein, 13 aa, Artificial
  Synthetic Peptide
CNLQLHNCQWGIC

SEQ ID NO: 107 - protein, 13 aa, Artificial
  Synthetic Peptide
  Xaa (2)..(2): Xaa is 3tBuTyr
CXLPDYLCGDEYC

SEQ ID NO: 108 - protein, 13 aa, Artificial
  Synthetic Peptide
  Xaa (6)..(6): Xaa is 3tBuTyr
CYLPDXLCGDEYC

SEQ ID NO: 109 - protein, 13 aa, Artificial
  Synthetic Peptide
  Xaa (12)..(12): Xaa is 3tBuTyr
CYLPDYLCGDEXC

SEQ ID NO: 110 - protein, 13 aa, Artificial
  Synthetic Peptide
  Xaa (2)..(2): Xaa is K(PYA)
CXLPDYLCGDEYC

SEQ ID NO: 111 - protein, 13 aa, Artificial
  Synthetic Peptide
  Xaa (5)..(5): Xaa is K(PYA)
CYLPXYLCGDEYC

SEQ ID NO: 112 - protein, 13 aa, Artificial
  Synthetic Peptide
  Xaa (9)..(9): Xaa is K(PYA)
CYLPDYLCXDEYC

SEQ ID NO: 113 - protein, 13 aa, Artificial
  Synthetic Peptide
  Xaa (11)..(11): Xaa is K(PYA)
CYLPDYLCGDXYC

SEQ ID NO: 114 - protein, 13 aa, Artificial
  Synthetic Peptide
  Xaa (12)..(12): Xaa is K(PYA)
CYLPDYLCGDEXC

SEQ ID NO: 115 - protein, 13 aa, Artificial
  Synthetic Peptide
  Xaa (9)..(9): Xaa is dK{PYA)
CYLPDYLCXDEYC

SEQ ID NO: 116 - protein, 13 aa, Artificial
  Synthetic Peptide
CALTTHNCQWGIC

SEQ ID NO: 117 - protein, 13 aa, Artificial
  Synthetic Peptide
CDLATHNCQWGIC

SEQ ID NO: 118 - protein, 13 aa, Artificial
  Synthetic Peptide
CDLTAHNCQWGIC

SEQ ID NO: 119 - protein, 13 aa, Artificial
  Synthetic Peptide
CDLTTHNCAWGIC

SEQ ID NO: 120 - protein, 13 aa, Artificial
  Synthetic Peptide
CDLTTHNCQWGAC

SEQ ID NO: 121 - protein, 13 aa, Artificial
  Synthetic Peptide
CNLTTHNCQWGIC

SEQ ID NO: 122 - protein, 13 aa, Artificial
  Synthetic Peptide
CDLQTHNCQWGIC

SEQ ID NO: 123 - protein, 13 aa, Artificial
  Synthetic Peptide
CDLTLHNCQWGIC

SEQ ID NO: 124 - protein, 13 aa, Artificial
  Synthetic Peptide
  Xaa (6)..(6): Xaa is His3Me
CDLTTXNCQWGIC

SEQ ID NO: 125 - protein, 13 aa, Artificial
  Synthetic Peptide
  Xaa (6)..(6): Xaa is 2Pal
CDLTTXNCQWGIC

SEQ ID NO: 126 - protein, 13 aa, Artificial
  Synthetic Peptide
  Xaa (6)..(6): Xaa is His1Me
CDLTTXNCQWGIC

SEQ ID NO: 127 - protein, 13 aa, Artificial
  Synthetic Peptide
  Xaa (6)..(6): Xaa is 4ThiAz
CDLTTXNCQWGIC

SEQ ID NO: 128 - protein, 13 aa, Artificial
  Synthetic Peptide
CDLTTHNCVWGIC

SEQ ID NO: 129 - protein, 13 aa, Artificial
  Synthetic Peptide
  misc_feature (9)..(9): Xaa can be any naturally occurring amino acid
CDLTTHNCXWGIC

SEQ ID NO: 130 - protein, 13 aa, Artificial
  Synthetic Peptide
  Xaa (10)..(10): Xaa is 1Nal
CDLTTHNCQXGIC

SEQ ID NO: 131 - protein, 13 aa, Artificial
  Synthetic Peptide
  Xaa (10)..(10): Xaa is Trp(Me)
CDLTTHNCQXGIC

SEQ ID NO: 132 - protein, 13 aa, Artificial
  Synthetic Peptide
  Xaa (12)..(12): Xaa is tBuGly
CDLTTHNCQWGXC

SEQ ID NO: 133 - protein, 13 aa, Artificial
  Synthetic Peptide
  Xaa (12)..(12): Xaa is tBuAla
CDLTTHNCQWGXC

SEQ ID NO: 134 - protein, 13 aa, Artificial
  Synthetic Peptide
  Xaa (12)..(12): Xaa is Chg
CDLTTHNCQWGXC

SEQ ID NO: 135 - protein, 13 aa, Artificial
  Synthetic Peptide
CDLTTHNCQWAIC

SEQ ID NO: 136 - protein, 13 aa, Artificial
  Synthetic Peptide
  Xaa (3)..(3): Xaa is Cba
CSXPDYLCADEYC

SEQ ID NO: 137 - protein, 13 aa, Artificial
  Synthetic Peptide
  Xaa (2)..(2): Xaa is HSer
  Xaa (3)..(3): Xaa is Cba
CXXPDYLCADEYC

SEQ ID NO: 138 - protein, 13 aa, Artificial
  Synthetic Peptide
  Xaa (3)..(3): Xaa is Cba
CNXPDYLCADEYC

SEQ ID NO: 139 - protein, 13 aa, Artificial
  Synthetic Peptide
  Xaa (2)..(2): Xaa is 4Pal
  Xaa (3)..(3): Xaa is Cba
CXXPDYLCADEYC

SEQ ID NO: 140 - protein, 13 aa, Artificial
  Synthetic Peptide
  Xaa (3)..(3): Xaa is Cba
  Xaa (4)..(4): Xaa is Cis-HyP
CYXXDYLCADEYC

SEQ ID NO: 141 - protein, 13 aa, Artificial
  Synthetic Peptide
  Xaa (3)..(3): Xaa is Cba
  Xaa (4)..(4): Xaa is NMeAla
CYXXDYLCADEYC

SEQ ID NO: 142 - protein, 13 aa, Artificial
  Synthetic Peptide
  Xaa (3)..(3): Xaa is Cba
CYXPNYLCADEYC

SEQ ID NO: 143 - protein, 13 aa, Artificial
  Synthetic Peptide
  Xaa (3)..(3): Xaa is Cba
CYXPQYLCADEYC

SEQ ID NO: 144 - protein, 13 aa, Artificial
  Synthetic Peptide
  Xaa (3)..(3): Xaa is Cba
CYXPDYLCVDEYC

SEQ ID NO: 145 - protein, 13 aa, Artificial
  Synthetic Peptide
  Xaa (3)..(3): Xaa is Cba
  Xaa (9)..(9): Xaa is dNva
CYXPDYLCXDEYC

SEQ ID NO: 146 - protein, 13 aa, Artificial
  Synthetic Peptide
  Xaa (3)..(3): Xaa is Cba
CYXPDYLCFDEYC

SEQ ID NO: 147 - protein, 13 aa, Artificial
  Synthetic Peptide
  Xaa (3)..(3): Xaa is Cba
  Xaa (9)..(9): Xaa is dCha
CYXPDYLCXDEYC

SEQ ID NO: 148 - protein, 13 aa, Artificial
  Synthetic Peptide
  Xaa (3)..(3): Xaa is Cba
  Xaa (9)..(9): Xaa is dK(PYA)
CYXPDYLCXDEYC

SEQ ID NO: 149 - protein, 13 aa, Artificial
  Synthetic Peptide
  Xaa (3)..(3): Xaa is Cba
  Xaa (9)..(9): Xaa is dNle
CYXPDYLCXDEYC

SEQ ID NO: 150 - protein, 13 aa, Artificial
  Synthetic Peptide
  Xaa (3)..(3): Xaa is Cba
  Xaa (6)..(6): Xaa is DOPA
CYXPDXLCADEYC

SEQ ID NO: 151 - protein, 13 aa, Artificial
  Synthetic Peptide
  Xaa (3)..(3): Xaa is Cba
  Xaa (6)..(6): Xaa is 2FTyr
CYXPDXLCADEYC

SEQ ID NO: 152 - protein, 13 aa, Artificial
  Synthetic Peptide
  Xaa (3)..(3): Xaa is Cba
  Xaa (7)..(7): Xaa is Nle
CYXPDYXCADEYC

SEQ ID NO: 153 - protein, 13 aa, Artificial
  Synthetic Peptide
  Xaa (1)..(1): Xaa is Pen
  Xaa (3)..(3): Xaa is Cba
XYXPDYLCADEYC

SEQ ID NO: 154 - protein, 13 aa, Artificial
  Synthetic Peptide
  Xaa (3)..(3): Xaa is Cba
  Xaa (8)..(8): Xaa is Pen
CYXPDYLXADEYC

SEQ ID NO: 155 - protein, 13 aa, Artificial
  Synthetic Peptide
  Xaa (3)..(3): Xaa is Cba
  Xaa (13)..(13): Xaa is Pen
CYXPDYLCADEYX

SEQ ID NO: 156 - protein, 13 aa, Artificial
  Synthetic Peptide
  Xaa (3)..(3): Xaa is Cba
CYXPDYLCADEYC

SEQ ID NO: 157 - protein, 13 aa, Artificial
  Synthetic Peptide
  Xaa (3)..(3): Xaa is Cba
CYXPDYLCADEYC

SEQ ID NO: 158 - protein, 13 aa, Artificial
  Synthetic Peptide
  Xaa (10)..(10): Xaa is AzaTrp
CDLTTHNCQXGIC

SEQ ID NO: 159 - protein, 13 aa, Artificial
  Synthetic Peptide
  Xaa (10)..(10): Xaa is 2MeTrp
CDLTTHNCQXGIC

SEQ ID NO: 160 - protein, 13 aa, Artificial
  Synthetic Peptide
  Xaa (10)..(10): Xaa is 6MeTrp
CDLTTHNCQXGIC

SEQ ID NO: 161 - protein, 13 aa, Artificial
  Synthetic Peptide
  Xaa (10)..(10): Xaa is 7MeTrp
CDLTTHNCQXGIC

SEQ ID NO: 162 - protein, 13 aa, Artificial
  Synthetic Peptide
  Xaa (10)..(10): Xaa is 6FTrp
CDLTTHNCQXGIC

SEQ ID NO: 163 - protein, 13 aa, Artificial
  Synthetic Peptide
  Xaa (10)..(10): Xaa is 5FTrp
CDLTTHNCQXGIC

SEQ ID NO: 164 - protein, 13 aa, Artificial
  Synthetic Peptide
  Xaa (10)..(10): Xaa is Dht
CDLTTHNCQXGIC

SEQ ID NO: 165 - protein, 13 aa, Artificial
  Synthetic Peptide
  Xaa (6)..(6): Xaa is 2FuAla
CDLTTXNCQWGIC

SEQ ID NO: 166 - protein, 13 aa, Artificial
  Synthetic Peptide
  Xaa (12)..(12): Xaa is EPA
CDLTTHNCQWGXC

SEQ ID NO: 167 - protein, 13 aa, Artificial
  Synthetic Peptide
  Xaa (12)..(12): Xaa is Nle
CDLTTHNCQWGXC

SEQ ID NO: 168 - protein, 13 aa, Artificial
  Synthetic Peptide
  Xaa (12)..(12): Xaa is AlloIle
CDLTTHNCQWGXC

SEQ ID NO: 169 - protein, 12 aa, Artificial
  Synthetic Peptide
CPPAVYCHPLDC

SEQ ID NO: 170 - protein, 12 aa, Artificial
  Synthetic Peptide
CPPEVFCHPLDC

SEQ ID NO: 171 - protein, 12 aa, Artificial
  Synthetic Peptide
CPPEVYCHPLDC

SEQ ID NO: 172 - protein, 12 aa, Artificial
  Synthetic Peptide
CPPEVWCHPLDC

SEQ ID NO: 173 - protein, 12 aa, Artificial
  Synthetic Peptide
CPPQVYCHPLDC

SEQ ID NO: 174 - protein, 12 aa, Artificial
  Synthetic Peptide
CPPEVWCHPLDC

SEQ ID NO: 175 - protein, 13 aa, Artificial
  Synthetic Peptide
  Xaa (5)..(5): Xaa is tBuGly
CRWSXEDPCGAWC

SEQ ID NO: 176 - protein, 13 aa, Artificial
  Synthetic Peptide
  Xaa (8)..(8): Xaa is HyP
CRWSVEDXCGAWC

SEQ ID NO: 177 - protein, 13 aa, Artificial
  Synthetic Peptide
  Xaa (8)..(8): Xaa is Aze
CRWSVEDXCGAWC

SEQ ID NO: 178 - protein, 13 aa, Artificial
  Synthetic Peptide
CRWSVEDPCAAWC

SEQ ID NO: 179 - protein, 13 aa, Artificial
  Synthetic Peptide
  Xaa (7)..(7): Xaa is Gla
CRWSVEXPCGAWC

SEQ ID NO: 180 - protein, 13 aa, Artificial
  Synthetic Peptide
  Xaa (8)..(8): Xaa is Aze
CRWSVEDXCGAWC

SEQ ID NO: 181 - protein, 13 aa, Artificial
  Synthetic Peptide
CMWIRSDPCGAWC

SEQ ID NO: 182 - protein, 13 aa, Artificial
  Synthetic Peptide
CRWYPDDPCGAWC

SEQ ID NO: 183 - protein, 13 aa, Artificial
  Synthetic Peptide
CEWHISEPCGAWC

SEQ ID NO: 184 - protein, 13 aa, Artificial
  Synthetic Peptide
CNWHVYEPCGAWC

SEQ ID NO: 185 - protein, 13 aa, Artificial
  Synthetic Peptide
CRWHFSEPCGAWC

SEQ ID NO: 186 - protein, 13 aa, Artificial
  Synthetic Peptide
CRWNLDDPCGAWC

SEQ ID NO: 187 - protein, 13 aa, Artificial
  Synthetic Peptide
CMWIRSDPCGAWC

SEQ ID NO: 188 - protein, 13 aa, Artificial
  Synthetic Peptide
CRWYPDDPCGAWC

SEQ ID NO: 189 - protein, 13 aa, Artificial
  Synthetic Peptide
CEWHISEPCGAWC

SEQ ID NO: 190 - protein, 13 aa, Artificial
  Synthetic Peptide
CNWHVYEPCGAWC

SEQ ID NO: 191 - protein, 13 aa, Artificial
  Synthetic Peptide
CRWHFSEPCGAWC

SEQ ID NO: 192 - protein, 13 aa, Artificial
  Synthetic Peptide
CRWNLDDPCGAWC

SEQ ID NO: 193 - protein, 13 aa, Artificial
  Synthetic Peptide
  Xaa (3)..(3): Xaa is 2MeTrp
CRXSVEDPCGAWC

SEQ ID NO: 194 - protein, 13 aa, Artificial
  Synthetic Peptide
  Xaa (3)..(3): Xaa is 6MeTrp
CRXSVEDPCGAWC

SEQ ID NO: 195 - protein, 13 aa, Artificial
  Synthetic Peptide
  Xaa (3)..(3): Xaa is 6FTrp
CRXSVEDPCGAWC

SEQ ID NO: 196 - protein, 13 aa, Artificial
  Synthetic Peptide
  Xaa (3)..(3): Xaa is 5FTrp
CRXSVEDPCGAWC

SEQ ID NO: 197 - protein, 13 aa, Artificial
  Synthetic Peptide
  Xaa (3)..(3): Xaa is 6ClTrp
CRXSVEDPCGAWC

SEQ ID NO: 198 - protein, 13 aa, Artificial
  Synthetic Peptide
  Xaa (3)..(3): Xaa is Trp(S)
CRXSVEDPCGAWC

SEQ ID NO: 199 - protein, 13 aa, Artificial
  Synthetic Peptide
  Xaa (3)..(3): Xaa is AzaTrp
CRXSVEDPCGAWC

SEQ ID NO: 200 - protein, 13 aa, Artificial
  Synthetic Peptide
  Xaa (12)..(12): Xaa is 2MeTrp
CRWSVEDPCGAXC

SEQ ID NO: 201 - protein, 13 aa, Artificial
  Synthetic Peptide
  Xaa (12)..(12): Xaa is 6FTrp
CRWSVEDPCGAXC

SEQ ID NO: 202 - protein, 13 aa, Artificial
  Synthetic Peptide
  Xaa (12)..(12): Xaa is 5FTrp
CRWSVEDPCGAXC

SEQ ID NO: 203 - protein, 13 aa, Artificial
  Synthetic Peptide
  Xaa (12)..(12): Xaa is 4MeoTrp
CRWSVEDPCGAXC

SEQ ID NO: 204 - protein, 13 aa, Artificial
  Synthetic Peptide
  Xaa (12)..(12): Xaa is 5MeoTrp
CRWSVEDPCGAXC

SEQ ID NO: 205 - protein, 13 aa, Artificial
  Synthetic Peptide
  Xaa (12)..(12): Xaa is Trp(S)
CRWSVEDPCGAXC

SEQ ID NO: 206 - protein, 13 aa, Artificial
  Synthetic Peptide
  Xaa (12)..(12): Xaa is DOPA
CRWSVEDPCGAXC

SEQ ID NO: 207 - protein, 13 aa, Artificial
  Synthetic Peptide
CRWYPDDPCGAWC

SEQ ID NO: 208 - protein, 13 aa, Artificial
  Synthetic Peptide
CRWHFSEPCGAWC

SEQ ID NO: 209 - protein, 13 aa, Artificial
  Synthetic Peptide
  Xaa (3)..(3): Xaa is 2MeTrp
CRXHFSEPCGAWC

SEQ ID NO: 210 - protein, 13 aa, Artificial
  Synthetic Peptide
CRWYFSEPCGAWC

SEQ ID NO: 211 - protein, 13 aa, Artificial
  Synthetic Peptide
CRWSFSEPCGAWC

SEQ ID NO: 212 - protein, 13 aa, Artificial
  Synthetic Peptide
CRWHPSEPCGAWC

SEQ ID NO: 213 - protein, 13 aa, Artificial
  Synthetic Peptide
CRWYPSEPCGAWC

SEQ ID NO: 214 - protein, 13 aa, Artificial
  Synthetic Peptide
CRWHPDEPCGAWC

SEQ ID NO: 215 - protein, 13 aa, Artificial
  Synthetic Peptide
CRWHPEEPCGAWC

SEQ ID NO: 216 - protein, 13 aa, Artificial
  Synthetic Peptide
CRWHFDEPCGAWC

SEQ ID NO: 217 - protein, 13 aa, Artificial
  Synthetic Peptide
CRWHFDDPCGAWC

SEQ ID NO: 218 - protein, 13 aa, Artificial
  Synthetic Peptide
CRWYFDEPCGAWC

SEQ ID NO: 219 - protein, 13 aa, Artificial
  Synthetic Peptide
  Xaa (4)..(4): Xaa is His1Me
CRWXFSEPCGAWC

SEQ ID NO: 220 - protein, 13 aa, Artificial
  Synthetic Peptide
  Xaa (4)..(4): Xaa is His3Me
CRWXFSEPCGAWC

SEQ ID NO: 221 - protein, 13 aa, Artificial
  Synthetic Peptide
  Xaa (4)..(4): Xaa is 4MeoPhe
CRWXFSEPCGAWC

SEQ ID NO: 222 - protein, 13 aa, Artificial
  Synthetic Peptide
  Xaa (4)..(4): Xaa is DOPA
CRWXFSEPCGAWC

SEQ ID NO: 223 - protein, 13 aa, Artificial
  Synthetic Peptide
  Xaa (4)..(4): Xaa is 26DiMeTyr
CRWXFSEPCGAWC

SEQ ID NO: 224 - protein, 13 aa, Artificial
  Synthetic Peptide
  Xaa (4)..(4): Xaa is 3BuTyr
CRWXFSEPCGAWC

SEQ ID NO: 225 - protein, 13 aa, Artificial
  Synthetic Peptide
  Xaa (4)..(4): Xaa is 4FPhe
CRWXFSEPCGAWC

SEQ ID NO: 226 - protein, 13 aa, Artificial
  Synthetic Peptide
  Xaa (5)..(5): Xaa is 4MePhe
CRWHXSEPCGAWC

SEQ ID NO: 227 - protein, 13 aa, Artificial
  Synthetic Peptide
  Xaa (5)..(5): Xaa is Aze
CRWHXSEPCGAWC

SEQ ID NO: 228 - protein, 13 aa, Artificial
  Synthetic Peptide
  Xaa (5)..(5): Xaa is HyP
CRWHXSEPCGAWC

SEQ ID NO: 229 - protein, 13 aa, Artificial
  Synthetic Peptide
  Xaa (5)..(5): Xaa is 4tBuPhe
CRWHXSEPCGAWC

SEQ ID NO: 230 - protein, 13 aa, Artificial
  Synthetic Peptide
  Xaa (5)..(5): Xaa is HPhe
CRWHXSEPCGAWC

SEQ ID NO: 231 - protein, 13 aa, Artificial
  Synthetic Peptide
  Xaa (5)..(5): Xaa is 4PhePro
CRWHXSEPCGAWC

SEQ ID NO: 232 - protein, 13 aa, Artificial
  Synthetic Peptide
  Xaa (6)..(6): Xaa is HSer
CRWHFXEPCGAWC

SEQ ID NO: 233 - protein, 13 aa, Artificial
  Synthetic Peptide
  Xaa (7)..(7): Xaa is Gla
CRWHFSXPCGAWC

SEQ ID NO: 234 - protein, 13 aa, Artificial
  Synthetic Peptide
  Xaa (7)..(7): Xaa is HGlu
CRWHFSXPCGAWC

SEQ ID NO: 235 - protein, 13 aa, Artificial
  Synthetic Peptide
CRWHFSEPCAAWC

SEQ ID NO: 236 - protein, 13 aa, Artificial
  Synthetic Peptide
  Xaa (8)..(8): Xaa is Aze
CRWYFSEXCAAWC

SEQ ID NO: 237 - protein, 13 aa, Artificial
  Synthetic Peptide
  Xaa (8)..(8): Xaa is Aze
CRWHFDEXCAAWC

SEQ ID NO: 238 - protein, 13 aa, Artificial
  Synthetic Peptide
  Xaa (8)..(8): Xaa is Aze
CRWYPSEXCAAWC

SEQ ID NO: 239 - protein, 13 aa, Artificial
  Synthetic Peptide
  Xaa (2)..(2): Xaa is HArg
CXWHFSEPCGAWC

SEQ ID NO: 240 - protein, 13 aa, Artificial
  Synthetic Peptide
  Xaa (5)..(5): Xaa is Cis-HyP
CRWHXSEPCGAWC

SEQ ID NO: 241 - protein, 13 aa, Artificial
  Synthetic Peptide
CRWHFSEPCGAWC

SEQ ID NO: 242 - protein, 13 aa, Artificial
  Synthetic Peptide
CRWHFSEPCGAWC

SEQ ID NO: 243 - protein, 13 aa, Artificial
  Synthetic Peptide
CRWHFSEPCGAWC

SEQ ID NO: 244 - protein, 14 aa, Artificial
  Synthetic Peptide
CVGLLELGPCSDLC

SEQ ID NO: 245 - protein, 14 aa, Artificial
  Synthetic Peptide
CPGLEELGPCSDLC

SEQ ID NO: 246 - protein, 14 aa, Artificial
  Synthetic Peptide
CVALEELGPCSDLC

SEQ ID NO: 247 - protein, 14 aa, Artificial
  Synthetic Peptide
  Xaa (4)..(4): Xaa is tBuAla
CVGXEELGPCSDLC

SEQ ID NO: 248 - protein, 14 aa, Artificial
  Synthetic Peptide
  Xaa (4)..(4): Xaa is Cba
CVGXEELGPCSDLC

SEQ ID NO: 249 - protein, 14 aa, Artificial
  Synthetic Peptide
CVGFEELGPCSDLC

SEQ ID NO: 250 - protein, 14 aa, Artificial
  Synthetic Peptide
  Xaa (4)..(4): Xaa is 1Nal
CVGXEELGPCSDLC

SEQ ID NO: 251 - protein, 14 aa, Artificial
  Synthetic Peptide
  Xaa (4)..(4): Xaa is 2Nal
CVGXEELGPCSDLC

SEQ ID NO: 252 - protein, 14 aa, Artificial
  Synthetic Peptide
CVGLPELGPCSDLC

SEQ ID NO: 253 - protein, 14 aa, Artificial
  Synthetic Peptide
  Xaa (5)..(5): Xaa is tBuAla
CVGLXELGPCSDLC

SEQ ID NO: 254 - protein, 14 aa, Artificial
  Synthetic Peptide
  Xaa (5)..(5): Xaa is Cba
CVGLXELGPCSDLC

SEQ ID NO: 255 - protein, 14 aa, Artificial
  Synthetic Peptide
  Xaa (5)..(5): Xaa is Cha
CVGLXELGPCSDLC

SEQ ID NO: 256 - protein, 14 aa, Artificial
  Synthetic Peptide
  Xaa (5)..(5): Xaa is Nle
CVGLXELGPCSDLC

SEQ ID NO: 257 - protein, 14 aa, Artificial
  Synthetic Peptide
  Xaa (6)..(6): Xaa is Gla
CVGLEXLGPCSDLC

SEQ ID NO: 258 - protein, 14 aa, Artificial
  Synthetic Peptide
  Xaa (9)..(9): Xaa is Aze
CVGLEELGXCSDLC

SEQ ID NO: 259 - protein, 14 aa, Artificial
  Synthetic Peptide
  Xaa (13)..(13): Xaa is tBuAla
CVGLEELGPCSDXC

SEQ ID NO: 260 - protein, 14 aa, Artificial
  Synthetic Peptide
  Xaa (13)..(13): Xaa is Cba
CVGLEELGPCSDXC

SEQ ID NO: 261 - protein, 14 aa, Artificial
  Synthetic Peptide
  Xaa (13)..(13): Xaa is Cha
CVGLEELGPCSDXC

SEQ ID NO: 262 - protein, 14 aa, Artificial
  Synthetic Peptide
  Xaa (4)..(4): Xaa is HLeu
CVGXEELGPCSDLC

SEQ ID NO: 263 - protein, 14 aa, Artificial
  Synthetic Peptide
  Xaa (5)..(5): Xaa is HLeu
CVGLXELGPCSDLC

SEQ ID NO: 264 - protein, 14 aa, Artificial
  Synthetic Peptide
  Xaa (6)..(6): Xaa is HGlu
CVGLEXLGPCSDLC

SEQ ID NO: 265 - protein, 15 aa, Artificial
  Synthetic Peptide
CTWPYCKSWGDVQDC

SEQ ID NO: 266 - protein, 12 aa, Artificial
  Synthetic Peptide
CDWWDPGCTYFC

SEQ ID NO: 267 - protein, 13 aa, Artificial
  Synthetic Peptide
  Xaa (5)..(5): Xaa is 4BnPro
CRWHXSEPCGAWC

SEQ ID NO: 268 - protein, 13 aa, Artificial
  Synthetic Peptide
  Xaa (5)..(5): Xaa is HPhe
  Xaa (8)..(8): Xaa is Aze
CRWHXSEXCGAWC